European Patent Specification EP 4 192 246 B1, published January 8, 2025. Title: PLANT PATHOGEN DEFENCE ELICITORS. Applicant: Université Libre de Bruxelles. The sequence listing filed with the application follows.

SEQUENCE LISTING (3 sequences)

SEQ ID NO: 1 - DNA, 678 bp, artificial sequence
  TtAA9E from Thielavia terrestris
atgttagctaatggtgcaatcgttttccttgctgccgccttgggtgtgtccggacattacacctggccacgtgtcaatgacggtgccgactggcagcaggtaaggaaggccgataattggcaggataacggttacgttggtgatgtgacgtcaccacaaatcaggtgctttcaagctaccccaagtcctgctccaagtgtacttaatactacagctggctctaccgtcacttactgggccaacccagatgtgtatcatccaggtcctgttcaattttacatggctagggtgcctgacggcgaagatattaactcatggaacggtgacggagctgtttggttcaaagtctacgaagatcatcctactttcggtgcccaattgacatggccttccactggtaagagttcttttgctgtacccattccaccatgcatcaaaagtggatattatctattgagagccgaacagattggattgcatgtggctcagagtgttggaggagctcaattctatatttcctgcgcccaattatctgttactggaggaggatcaaccgaaccacccaataaggttgcattccccggagcttattccgccactgatccaggtattcttattaatatttattatcctgtgcctacgtcctatcaaaatcctggaccagctgtattttcttgc

SEQ ID NO: 2 - DNA, 40 bp, artificial sequence
  MtAA9A forward primer
agcatcattacacctcagcaatgaagtccttcaccctcac

SEQ ID NO: 3 - DNA, 40 bp, artificial sequence
  MtAA9A reverse primer
taaatcactagatatctctattagacgcactgcgagtagt